European Patent Specification EP 3 801 473 B1, published April 2, 2025. Title: SETBP1 Inhibitors for the Treatment of Myeloid Neoplasms and Solid Tumors. Applicant: Du, Yang Nguyen, Nhu The Henry M. Jackson Foundation for the Advancement of Military Medicine, Inc. The sequence listing filed with the application follows.

SEQUENCE LISTING (1 sequence)

SEQ ID NO: 1 - protein, 240 aa, Artificial Sequence
  Synthetic
MGSSHHHHHHSSGLVPKGSHMLEESHSEETIPSDSGIGTDNNSTSDQAEKSSESRRRYSFDFCSLDNPEAIPSDTSTKNRHGHRQKHLIVDTFLAHESLKKPKHKRKRKSLQNRDDLQFLAELEELITKFQVFRISHRGYTFYHENPYPSIFRINFDQYYPVPYIQYDPLLYLRRTSDLKSKKKRGRPAKTNDTMTKVPFLQGFSYPIPSGSYYAPYGMPYTSMPMMNLGYYGQYPAPLY